European Patent Application EP 4 350 708 A1, published April 10, 2024. Title: Method for diagnosing and predicting cancer type using fragment end motif frequency and size of cell-free nucleic acid. Applicant: Green Cross Genome Corporation University of Ulsan Foundation For Industry Cooperation THE ASAN FOUNDATION. The sequence listing filed with the application follows.

SEQUENCE LISTING (4 sequences)

SEQ ID NO: 1 - DNA, 15 bp, Artificial Sequence
  forward 1
tacagactttggaat

SEQ ID NO: 2 - DNA, 15 bp, Artificial Sequence
  reverse 1
atgactgaaacctta

SEQ ID NO: 3 - DNA, 18 bp, Artificial Sequence
  forward 2
tacagactagtttggaat

SEQ ID NO: 4 - DNA, 18 bp, Artificial Sequence
  reverse 2
atgactgatcaaacctta